European Patent Application EP 4 455 295 A1, published October 30, 2024. Title: Gene therapy for the treatment of Glutaric Aciduria type I. Applicant: FUNDACIÓ DE RECERCA CLÍNIC BARCELONA-INSTITUT D'INVESTIGACIONS BIOMÈDIQUES AUGUST PI I SUNYER. The sequence listing filed with the application follows.

SEQUENCE LISTING (12 sequences)

SEQ ID NO: 1 - DNA, 304 bp, synthetic construct
  source 1..304: mol_type = other DNA
cgttacataacttacggtaaatggcccgcctggctgaccgcccaacgacccccgcccattgacgtcaataatgacgtatgttcccatagtaacgccaatagggactttccattgacgtcaatgggtggactatttacggtaaactgcccacttggcagtacatcaagtgtatcatatgccaagtacgccccctattgacgtcaatgacggtaaatggcccgcctggcattatgcccagtacatgaccttatgggactttcctacttggcagtacatctacgtattagtcatcgctattaccatg

SEQ ID NO: 2 - DNA, 276 bp, synthetic construct
  source 1..276: mol_type = other DNA
tcgaggtgagccccacgttctgcttcactctccccatctcccccccctccccacccccaattttgtatttatttattttttaattattttgtgcagcgatgggggcggggggggggggggcgcgcgccaggcggggcggggcggggcgaggggcggggcggggcgaggcggagaggtgcggcggcagccaatcagagcggcgcgctccgaaagtttccttttatggcgaggcggcggcggcggcggccctataaaaagcgaagcgcgcggcgggcg

SEQ ID NO: 3 - DNA, 1012 bp, synthetic construct
  source 1..1012: mol_type = other DNA
ggagtcgctgcgttgccttcgccccgtgccccgctccgcgccgcctcgcgccgcccgccccggctctgactgaccgcgttactcccacaggtgagcgggcgggacggcccttctcctccgggctgtaattagcgcttggtttaatgacggctcgtttcttttctgtggctgcgtgaaagccttaaagggctccgggagggccctttgtgcgggggggagcggctcggggggtgcgtgcgtgtgtgtgtgcgtggggagcgccgcgtgcggcccgcgctgcccggcggctgtgagcgctgcgggcgcggcgcggggctttgtgcgctccgcgtgtgcgcgaggggagcgcggccgggggcggtgccccgcggtgcgggggggctgcgaggggaacaaaggctgcgtgcggggtgtgtgcgtgggggggtgagcagggggtgtgggcgcggcggtcgggctgtaacccccccctgcacccccctccccgagttgctgagcacggcccggcttcgggtgcggggctccgtacggggcgtggcgcggggctcgccgtgccgggcggggggtggcggcaggtgggggtgccgggcggggcggggccgcctcgggccggggagggctcgggggaggggcgcggcggccccggagcgccggcggctgtcgaggcgcggcgagccgcagccattgccttttatggtaatcgtgcgagagggcgcagggacttcctttgtcccaaatctgtgcggagccgaaatctgggaggcgccgccgcaccccctctagcgggcgcggggcgaagcggtgcggcgccggcaggaaggaaatgggcggggagggccttcgtgcgtcgccgcgccgccgtccccttctccctctccagcctcggggctgtccgcggggggacggctgccttcgggggggacggggcagggcggggttcggcttctggcgtgtgaccggcggctctagagcctctgctaaccatgttcatgccttcttctttttcctacag

SEQ ID NO: 4 - DNA, 1592 bp, synthetic construct
  source 1..1592: mol_type = other DNA
cgttacataacttacggtaaatggcccgcctggctgaccgcccaacgacccccgcccattgacgtcaataatgacgtatgttcccatagtaacgccaatagggactttccattgacgtcaatgggtggactatttacggtaaactgcccacttggcagtacatcaagtgtatcatatgccaagtacgccccctattgacgtcaatgacggtaaatggcccgcctggcattatgcccagtacatgaccttatgggactttcctacttggcagtacatctacgtattagtcatcgctattaccatgtcgaggtgagccccacgttctgcttcactctccccatctcccccccctccccacccccaattttgtatttatttattttttaattattttgtgcagcgatgggggcggggggggggggggcgcgcgccaggcggggcggggcggggcgaggggcggggcggggcgaggcggagaggtgcggcggcagccaatcagagcggcgcgctccgaaagtttccttttatggcgaggcggcggcggcggcggccctataaaaagcgaagcgcgcggcgggcgggagtcgctgcgttgccttcgccccgtgccccgctccgcgccgcctcgcgccgcccgccccggctctgactgaccgcgttactcccacaggtgagcgggcgggacggcccttctcctccgggctgtaattagcgcttggtttaatgacggctcgtttcttttctgtggctgcgtgaaagccttaaagggctccgggagggccctttgtgcgggggggagcggctcggggggtgcgtgcgtgtgtgtgtgcgtggggagcgccgcgtgcggcccgcgctgcccggcggctgtgagcgctgcgggcgcggcgcggggctttgtgcgctccgcgtgtgcgcgaggggagcgcggccgggggcggtgccccgcggtgcgggggggctgcgaggggaacaaaggctgcgtgcggggtgtgtgcgtgggggggtgagcagggggtgtgggcgcggcggtcgggctgtaacccccccctgcacccccctccccgagttgctgagcacggcccggcttcgggtgcggggctccgtacggggcgtggcgcggggctcgccgtgccgggcggggggtggcggcaggtgggggtgccgggcggggcggggccgcctcgggccggggagggctcgggggaggggcgcggcggccccggagcgccggcggctgtcgaggcgcggcgagccgcagccattgccttttatggtaatcgtgcgagagggcgcagggacttcctttgtcccaaatctgtgcggagccgaaatctgggaggcgccgccgcaccccctctagcgggcgcggggcgaagcggtgcggcgccggcaggaaggaaatgggcggggagggccttcgtgcgtcgccgcgccgccgtccccttctccctctccagcctcggggctgtccgcggggggacggctgccttcgggggggacggggcagggcggggttcggcttctggcgtgtgaccggcggctctagagcctctgctaaccatgttcatgccttcttctttttcctacag

SEQ ID NO: 5 - DNA, 1320 bp, synthetic construct
  source 1..1320: mol_type = other DNA
atggccctgagaggcgtctccgtgcggctgctgagccgcggacccggcctgcacgtccttcgcacgtgggtctcgtcggcggcgcagaccgagaaaggcgggagaacacagagccaactggctaagtcctcgcgtcccgagtttgactggcaggacccgctggtgctggaggagcagctgaccacagatgagatcctcatcagggacaccttccgcacctactgccaggagagactcatgcctcgcatcctgttggccaatcgcaacgaagtttttcatcgggagatcatttcggagatgggggagttgggtgtgctgggccccaccatcaaaggatatggctgtgctggggtttcgtctgtggcctatgggctcctggcccgagagctggagcgggtggacagtggctacaggtcggcgatgagtgtccagtcctccctcgtcatgcaccctatctatgcctatggcagcgaggaacagcggcagaagtacctgccccagctggccaagggggagctcctgggctgcttcgggctcacagagcccaacagcggaagtgaccccagcagcatggagaccagagcccactacaactcatccaacaagagctacaccctcaatgggaccaagacctggatcacgaactcgcctatggccgatctgtttgtagtgtgggctcggtgtgaagatggctgcattcggggcttcctgctggagaaggggatgcggggtctctcggcccccaggatccagggcaagttctcgctgcgggcctcagccacaggcatgatcatcatggacggtgtggaggtgccagaggagaatgtgctccctggtgcatccagcctggggggtcccttcggctgcctgaacaacgcccggtacggcatcgcgtggggcgtgcttggagcttcggagttctgcttgcacacagcccggcagtacgccctcgacaggatgcagtttggtgtcccactggccaggaaccagctgattcagaagaagctggcagacatgctcactgagattaccctgggccttcacgcctgcctgcagctcggccgcttgaaggaccaggacaaggctgcccccgagatggtttctctgctgaagaggaataactgtgggaaagccctggacatcgcccgccaggcccgagacatgctgggggggaatgggatttctgacgagtatcacgtgatccggcacgccatgaacctggaggccgtgaacacctacgaaggtacacatgacattcacgccctgatccttgggagagctatcacgggaatccaggcgttcacggccagcaagttgtga

SEQ ID NO: 6 - DNA, 589 bp, synthetic construct
  source 1..589: mol_type = other DNA
aatcaacctctggattacaaaatttgtgaaagattgactggtattcttaactatgttgctccttttacgctatgtggatacgctgctttaatgcctttgtatcatgctattgcttcccgtatggctttcattttctcctccttgtataaatcctggttgctgtctctttatgaggagttgtggcccgttgtcaggcaacgtggcgtggtgtgcactgtgtttgctgacgcaacccccactggttggggcattgccaccacctgtcagctcctttccgggactttcgctttccccctccctattgccacggcggaactcatcgccgcctgccttgcccgctgctggacaggggctcggctgttgggcactgacaattccgtggtgttgtcggggaaatcatcgtcctttccttggctgctcgcctatgttgccacctggattctgcgcgggacgtccttctgctacgtcccttcggccctcaatccagcggaccttccttcccgcggcctgctgccggctctgcggcctcttccgcgtcttcgccttcgccctcagacgagtcggatctccctttgggccgcctccccgc

SEQ ID NO: 7 - DNA, 477 bp, synthetic construct
  source 1..477: mol_type = other DNA
gggtggcatccctgtgacccctccccagtgcctctcctggccctggaagttgccactccagtgcccaccagccttgtcctaataaaattaagttgcatcattttgtctgactaggtgtccttctataatattatggggtggaggggggtggtatggagcaaggggcaagttgggaagacaacctgtagggcctgcggggtctattgggaaccaagctggagtgcagtggcacaatcttggctcactgcaatctccgcctcctgggttcaagcgattctcctgcctcagcctcccgagttgttgggattccaggcatgcatgaccaggctcagctaatttttgtttttttggtagagacggggtttcaccatattggccaggctggtctccaactcctaatctcaggtgatctacccaccttggcctcccaaattgctgggattacaggcgtgaaccactgctcccttccctgtcctt

SEQ ID NO: 8 - DNA, 141 bp, synthetic construct
  source 1..141: mol_type = other DNA
cctgcaggcagctgcgcgctcgctcgctcactgaggccgcccgggcaaagcccgggcgtcgggcgacctttggtcgcccggcctcagtgagcgagcgagcgcgcagagagggagtggccaactccatcactaggggttcct

SEQ ID NO: 9 - DNA, 4006 bp, synthetic construct
  source 1..4006: mol_type = other DNA
cgttacataacttacggtaaatggcccgcctggctgaccgcccaacgacccccgcccattgacgtcaataatgacgtatgttcccatagtaacgccaatagggactttccattgacgtcaatgggtggactatttacggtaaactgcccacttggcagtacatcaagtgtatcatatgccaagtacgccccctattgacgtcaatgacggtaaatggcccgcctggcattatgcccagtacatgaccttatgggactttcctacttggcagtacatctacgtattagtcatcgctattaccatgtcgaggtgagccccacgttctgcttcactctccccatctcccccccctccccacccccaattttgtatttatttattttttaattattttgtgcagcgatgggggcggggggggggggggcgcgcgccaggcggggcggggcggggcgaggggcggggcggggcgaggcggagaggtgcggcggcagccaatcagagcggcgcgctccgaaagtttccttttatggcgaggcggcggcggcggcggccctataaaaagcgaagcgcgcggcgggcgggagtcgctgcgttgccttcgccccgtgccccgctccgcgccgcctcgcgccgcccgccccggctctgactgaccgcgttactcccacaggtgagcgggcgggacggcccttctcctccgggctgtaattagcgcttggtttaatgacggctcgtttcttttctgtggctgcgtgaaagccttaaagggctccgggagggccctttgtgcgggggggagcggctcggggggtgcgtgcgtgtgtgtgtgcgtggggagcgccgcgtgcggcccgcgctgcccggcggctgtgagcgctgcgggcgcggcgcggggctttgtgcgctccgcgtgtgcgcgaggggagcgcggccgggggcggtgccccgcggtgcgggggggctgcgaggggaacaaaggctgcgtgcggggtgtgtgcgtgggggggtgagcagggggtgtgggcgcggcggtcgggctgtaacccccccctgcacccccctccccgagttgctgagcacggcccggcttcgggtgcggggctccgtacggggcgtggcgcggggctcgccgtgccgggcggggggtggcggcaggtgggggtgccgggcggggcggggccgcctcgggccggggagggctcgggggaggggcgcggcggccccggagcgccggcggctgtcgaggcgcggcgagccgcagccattgccttttatggtaatcgtgcgagagggcgcagggacttcctttgtcccaaatctgtgcggagccgaaatctgggaggcgccgccgcaccccctctagcgggcgcggggcgaagcggtgcggcgccggcaggaaggaaatgggcggggagggccttcgtgcgtcgccgcgccgccgtccccttctccctctccagcctcggggctgtccgcggggggacggctgccttcgggggggacggggcagggcggggttcggcttctggcgtgtgaccggcggctctagagcctctgctaaccatgttcatgccttcttctttttcctacagaagcttcgaattctgcagtcgacatggccctgagaggcgtctccgtgcggctgctgagccgcggacccggcctgcacgtccttcgcacgtgggtctcgtcggcggcgcagaccgagaaaggcgggagaacacagagccaactggctaagtcctcgcgtcccgagtttgactggcaggacccgctggtgctggaggagcagctgaccacagatgagatcctcatcagggacaccttccgcacctactgccaggagagactcatgcctcgcatcctgttggccaatcgcaacgaagtttttcatcgggagatcatttcggagatgggggagttgggtgtgctgggccccaccatcaaaggatatggctgtgctggggtttcgtctgtggcctatgggctcctggcccgagagctggagcgggtggacagtggctacaggtcggcgatgagtgtccagtcctccctcgtcatgcaccctatctatgcctatggcagcgaggaacagcggcagaagtacctgccccagctggccaagggggagctcctgggctgcttcgggctcacagagcccaacagcggaagtgaccccagcagcatggagaccagagcccactacaactcatccaacaagagctacaccctcaatgggaccaagacctggatcacgaactcgcctatggccgatctgtttgtagtgtgggctcggtgtgaagatggctgcattcggggcttcctgctggagaaggggatgcggggtctctcggcccccaggatccagggcaagttctcgctgcgggcctcagccacaggcatgatcatcatggacggtgtggaggtgccagaggagaatgtgctccctggtgcatccagcctggggggtcccttcggctgcctgaacaacgcccggtacggcatcgcgtggggcgtgcttggagcttcggagttctgcttgcacacagcccggcagtacgccctcgacaggatgcagtttggtgtcccactggccaggaaccagctgattcagaagaagctggcagacatgctcactgagattaccctgggccttcacgcctgcctgcagctcggccgcttgaaggaccaggacaaggctgcccccgagatggtttctctgctgaagaggaataactgtgggaaagccctggacatcgcccgccaggcccgagacatgctgggggggaatgggatttctgacgagtatcacgtgatccggcacgccatgaacctggaggccgtgaacacctacgaaggtacacatgacattcacgccctgatccttgggagagctatcacgggaatccaggcgttcacggccagcaagttgtgaagcttaatcaacctctggattacaaaatttgtgaaagattgactggtattcttaactatgttgctccttttacgctatgtggatacgctgctttaatgcctttgtatcatgctattgcttcccgtatggctttcattttctcctccttgtataaatcctggttgctgtctctttatgaggagttgtggcccgttgtcaggcaacgtggcgtggtgtgcactgtgtttgctgacgcaacccccactggttggggcattgccaccacctgtcagctcctttccgggactttcgctttccccctccctattgccacggcggaactcatcgccgcctgccttgcccgctgctggacaggggctcggctgttgggcactgacaattccgtggtgttgtcggggaaatcatcgtcctttccttggctgctcgcctatgttgccacctggattctgcgcgggacgtccttctgctacgtcccttcggccctcaatccagcggaccttccttcccgcggcctgctgccggctctgcggcctcttccgcgtcttcgccttcgccctcagacgagtcggatctccctttgggccgcctccccgcgggtggcatccctgtgacccctccccagtgcctctcctggccctggaagttgccactccagtgcccaccagccttgtcctaataaaattaagttgcatcattttgtctgactaggtgtccttctataatattatggggtggaggggggtggtatggagcaaggggcaagttgggaagacaacctgtagggcctgcggggtctattgggaaccaagctggagtgcagtggcacaatcttggctcactgcaatctccgcctcctgggttcaagcgattctcctgcctcagcctcccgagttgttgggattccaggcatgcatgaccaggctcagctaatttttgtttttttggtagagacggggtttcaccatattggccaggctggtctccaactcctaatctcaggtgatctacccaccttggcctcccaaattgctgggattacaggcgtgaaccactgctcccttccctgtcctt

SEQ ID NO: 10 - DNA, 1348 bp, synthetic construct
  source 1..1348: mol_type = other DNA
aagcttcgaattctgcagtcgacatggccctgagaggcgtctccgtgcggctgctgagccgcggacccggcctgcacgtccttcgcacgtgggtctcgtcggcggcgcagaccgagaaaggcgggagaacacagagccaactggctaagtcctcgcgtcccgagtttgactggcaggacccgctggtgctggaggagcagctgaccacagatgagatcctcatcagggacaccttccgcacctactgccaggagagactcatgcctcgcatcctgttggccaatcgcaacgaagtttttcatcgggagatcatttcggagatgggggagttgggtgtgctgggccccaccatcaaaggatatggctgtgctggggtttcgtctgtggcctatgggctcctggcccgagagctggagcgggtggacagtggctacaggtcggcgatgagtgtccagtcctccctcgtcatgcaccctatctatgcctatggcagcgaggaacagcggcagaagtacctgccccagctggccaagggggagctcctgggctgcttcgggctcacagagcccaacagcggaagtgaccccagcagcatggagaccagagcccactacaactcatccaacaagagctacaccctcaatgggaccaagacctggatcacgaactcgcctatggccgatctgtttgtagtgtgggctcggtgtgaagatggctgcattcggggcttcctgctggagaaggggatgcggggtctctcggcccccaggatccagggcaagttctcgctgcgggcctcagccacaggcatgatcatcatggacggtgtggaggtgccagaggagaatgtgctccctggtgcatccagcctggggggtcccttcggctgcctgaacaacgcccggtacggcatcgcgtggggcgtgcttggagcttcggagttctgcttgcacacagcccggcagtacgccctcgacaggatgcagtttggtgtcccactggccaggaaccagctgattcagaagaagctggcagacatgctcactgagattaccctgggccttcacgcctgcctgcagctcggccgcttgaaggaccaggacaaggctgcccccgagatggtttctctgctgaagaggaataactgtgggaaagccctggacatcgcccgccaggcccgagacatgctgggggggaatgggatttctgacgagtatcacgtgatccggcacgccatgaacctggaggccgtgaacacctacgaaggtacacatgacattcacgccctgatccttgggagagctatcacgggaatccaggcgttcacggccagcaagttgtgaagctt

SEQ ID NO: 11 - protein, 439 aa, synthetic construct
MALRGVSVRLLSRGPGLHVLRTWVSSAAQTEKGGRTQSQLAKSSRPEFDWQDPLVLEEQLTTDEILIRDTFRTYCQERLMPRILLANRNEVFHREIISEMGELGVLGPTIKGYGCAGVSSVAYGLLARELERVDSGYRSAMSVQSSLVMHPIYAYGSEEQRQKYLPQLAKGELLGCFGLTEPNSGSDPSSMETRAHYNSSNKSYTLNGTKTWITNSPMADLFVVWARCEDGCIRGFLLEKGMRGLSAPRIQGKFSLRASATGMIIMDGVEVPEENVLPGASSLGGPFGCLNNARYGIAWGVLGASEFCLHTARQYALDRMQFGVPLARNQLIQKKLADMLTEITLGLHACLQLGRLKDQDKAAPEMVSLLKRNNCGKALDIARQARDMLGGNGISDEYHVIRHAMNLEAVNTYEGTHDIHALILGRAITGIQAFTASKL

SEQ ID NO: 12 - DNA, 141 bp, synthetic construct
  source 1..141: mol_type = other DNA
aggaacccctagtgatggagttggccactccctctctgcgcgctcgctcgctcactgaggccgggcgaccaaaggtcgcccgacgcccgggctttgcccgggcggcctcagtgagcgagcgagcgcgcagctgcctgcagg